European Patent Specification EP 3 651 817 B1, published May 3, 2023. Title: Tissue Scaffold. Applicant: RAFT Enterprises Ltd. The sequence listing filed with the application follows.

SEQUENCE LISTING (14 sequences)

SEQ ID NO: 1 - DNA, 21 bp, Artificial Sequence
  Synthetic primer
cgcctgagcaaagtaaatgag

SEQ ID NO: 2 - DNA, 19 bp, Artificial Sequence
  Synthetic primer
gccctcgatatagcggatg

SEQ ID NO: 3 - DNA, 25 bp, Artificial Sequence
  Synthetic primer
gaataaagatggggttctcatatcc

SEQ ID NO: 4 - DNA, 21 bp, Artificial Sequence
  Synthetic primer
aacttcagcaaactcaaactt

SEQ ID NO: 5 - DNA, 25 bp, Artificial Sequence
  Synthetic primer
cggcaactctagtatttaggataac

SEQ ID NO: 6 - DNA, 24 bp, Artificial Sequence
  Synthetic primer
caaataaaatgacaaggcacgatt

SEQ ID NO: 7 - DNA, 20 bp, Artificial Sequence
  Synthetic primer
ttctccccttttcccactga

SEQ ID NO: 8 - DNA, 25 bp, Artificial Sequence
  Synthetic primer
caaacgcaatcactatctataccat

SEQ ID NO: 9 - DNA, 19 bp, Artificial Sequence
  Synthetic primer
ggaccagtacccgcacttg

SEQ ID NO: 10 - DNA, 20 bp, Artificial Sequence
  Synthetic primer
aatccgggtggtccttcttg

SEQ ID NO: 11 - DNA, 23 bp, Artificial Sequence
  Synthetic primer
cactaaggaaggaattgggaaca

SEQ ID NO: 12 - DNA, 25 bp, Artificial Sequence
  Synthetic primer
gggattaaaatcaagagcatcattg

SEQ ID NO: 13 - DNA, 18 bp, Artificial Sequence
  Synthetic primer
cgtttcgtgtccctttca

SEQ ID NO: 14 - DNA, 25 bp, Artificial Sequence
  Synthetic primer
cctcttgttcattcttgttcgtatt